European Patent Specification EP 3 038 462 B1, published March 15, 2023. Title: METHOD FOR ENHANCING TUMOR GROWTH. Applicant: MINERVA BIOTECHNOLOGIES CORPORATION. Application 14835875.7. The sequence listing filed with the application follows.

SEQUENCE LISTING (146 sequences)

SEQ ID NO: 1 - protein, 1255 aa, Artificial Sequence
  full-length MUC1 Receptor
MTPGTQSPFFLLLLLTVLTVVTGSGHASSTPGGEKETSATQRSSVPSSTEKNAVSMTSSVLSSHSPGSGSSTTQGQDVTLAPATEPASGSAATWGQDVTSVPVTRPALGSTTPPAHDVTSAPDNKPAPGSTAPPAHGVTSAPDTRPAPGSTAPPAHGVTSAPDTRPAPGSTAPPAHGVTSAPDTRPAPGSTAPPAHGVTSAPDTRPAPGSTAPPAHGVTSAPDTRPAPGSTAPPAHGVTSAPDTRPAPGSTAPPAHGVTSAPDTRPAPGSTAPPAHGVTSAPDTRPAPGSTAPPAHGVTSAPDTRPAPGSTAPPAHGVTSAPDTRPAPGSTAPPAHGVTSAPDTRPAPGSTAPPAHGVTSAPDTRPAPGSTAPPAHGVTSAPDTRPAPGSTAPPAHGVTSAPDTRPAPGSTAPPAHGVTSAPDTRPAPGSTAPPAHGVTSAPDTRPAPGSTAPPAHGVTSAPDTRPAPGSTAPPAHGVTSAPDTRPAPGSTAPPAHGVTSAPDTRPAPGSTAPPAHGVTSAPDTRPAPGSTAPPAHGVTSAPDTRPAPGSTAPPAHGVTSAPDTRPAPGSTAPPAHGVTSAPDTRPAPGSTAPPAHGVTSAPDTRPAPGSTAPPAHGVTSAPDTRPAPGSTAPPAHGVTSAPDTRPAPGSTAPPAHGVTSAPDTRPAPGSTAPPAHGVTSAPDTRPAPGSTAPPAHGVTSAPDTRPAPGSTAPPAHGVTSAPDTRPAPGSTAPPAHGVTSAPDTRPAPGSTAPPAHGVTSAPDTRPAPGSTAPPAHGVTSAPDTRPAPGSTAPPAHGVTSAPDTRPAPGSTAPPAHGVTSAPDTRPAPGSTAPPAHGVTSAPDTRPAPGSTAPPAHGVTSAPDTRPAPGSTAPPAHGVTSAPDTRPAPGSTAPPAHGVTSAPDTRPAPGSTAPPAHGVTSAPDTRPAPGSTAPPAHGVTSAPDNRPALGSTAPPVHNVTSASGSASGSASTLVHNGTSARATTTPASKSTPFSIPSHHSDTPTTLASHSTKTDASSTHHSSVPPLTSSNHSTSPQLSTGVSFFFLSFHISNLQFNSSLEDPSTDYYQELQRDISEMFLQIYKQGGFLGLSNIKFRPGSVVVQLTLAFREGTINVHDVETQFNQYKTEAASRYNLTISDVSVSDVPFPFSAQSGAGVPGWGIALLVLVCVLVALAIVYLIALAVCQCRRKNYGQLDIFPARDTYHPMSEYPTYHTHGRYVPPSSTDRSPYEKVSAGNGGSSLSYTNPAVAAASANL

SEQ ID NO: 2 - protein, 19 aa, Artificial Sequence
  N-terminal MUC-1 signaling sequence
MTPGTQSPFFLLLLLTVLT

SEQ ID NO: 3 - protein, 23 aa, Artificial Sequence
  N-terminal MUC-1 signaling sequence
MTPGTQSPFFLLLLLTVLTVVTA

SEQ ID NO: 4 - protein, 23 aa, Artificial Sequence
  N-terminal MUC-1 signaling sequence
MTPGTQSPFFLLLLLTVLTVVTG

SEQ ID NO: 5 - protein, 146 aa, Artificial Sequence
  truncated MUC1 receptor isoform
GTINVHDVETQFNQYKTEAASRYNLTISDVSVSDVPFPFSAQSGAGVPGWGIALLVLVCVLVALAIVYLIALAVCQCRRKNYGQLDIFPARDTYHPMSEYPTYHTHGRYVPPSSTDRSPYEKVSAGNGGSSLSYTNPAVAAASANL

SEQ ID NO: 6 - protein, 45 aa, Artificial Sequence
  extracellular domain of Native Primary Sequence
GTINVHDVETQFNQYKTEAASRYNLTISDVSVSDVPFPFSAQSGA

SEQ ID NO: 7 - protein, 44 aa, Artificial Sequence
  extracellular domain of Native Primary Sequence
TINVHDVETQFNQYKTEAASRYNLTISDVSVSDVPFPFSAQSGA

SEQ ID NO: 8 - protein, 45 aa, Artificial Sequence
  extracellular domain of "SPY" functional variant
GTINVHDVETQFNQYKTEAASPYNLTISDVSVSDVPFPFSAQSGA

SEQ ID NO: 9 - protein, 44 aa, Artificial Sequence
  extracellular domain of "SPY" functional variant
TINVHDVETQFNQYKTEAASPYNLTISDVSVSDVPFPFSAQSGA

SEQ ID NO: 10 - DNA, 216 bp, Artificial Sequence
  MUC1 cytoplasmic domain nucleotide sequence
tgtcagtgccgccgaaagaactacgggcagctggacatctttccagcccgggatacctaccatcctatgagcgagtaccccacctaccacacccatgggcgctatgtgccccctagcagtaccgatcgtagcccctatgagaaggtttctgcaggtaacggtggcagcagcctctcttacacaaacccagcagtggcagccgcttctgccaacttg

SEQ ID NO: 11 - protein, 72 aa, Artificial Sequence
  MUC1 cytoplasmic domain amino acid sequence
CQCRRKNYGQLDIFPARDTYHPMSEYPTYHTHGRYVPPSSTDRSPYEKVSAGNGGSSLSYTNPAVAAASANL

SEQ ID NO: 12 - DNA, 854 bp, Artificial Sequence
  NME7 nucleotide sequence
gagatcctgagacaatgaatcatagtgaaagattcgttttcattgcagagtggtatgatccaaatgcttcacttcttcgacgttatgagcttttattttacccaggggatggatctgttgaaatgcatgatgtaaagaatcatcgcacctttttaaagcggaccaaatatgataacctgcacttggaagatttatttataggcaacaaagtgaatgtcttttctcgacaactggtattaattgactatggggatcaatatacagctcgccagctgggcagtaggaaagaaaaaacgctagccctaattaaaccagatgcaatatcaaaggctggagaaataattgaaataataaacaaagctggatttactataaccaaactcaaaatgatgatgctttcaaggaaagaagcattggattttcatgtagatcaccagtcaagaccctttttcaatgagctgatccagtttattacaactggtcctattattgccatggagattttaagagatgatgctatatgtgaatggaaaagactgctgggacctgcaaactctggagtggcacgcacagatgcttctgaaagcattagagccctctttggaacagatggcataagaaatgcagcgcatggccctgattcttttgcttctgcggccagagaaatggagttgttttttccttcaagtggaggttgtgggccggcaaacactgctaaatttactaattgtacctgttgcattgttaaaccccatgctgtcagtgaaggtatgttgaatacactatattcagtacattttgttaataggagagcaatgtttattttcttgatgtactttatgtatagaaaataa

SEQ ID NO: 13 - protein, 283 aa, Artificial Sequence
  NME7 amino acid sequence
DPETMNHSERFVFIAEWYDPNASLLRRYELLFYPGDGSVEMHDVKNHRTFLKRTKYDNLHLEDLFIGNKVNVFSRQLVLIDYGDQYTARQLGSRKEKTLALIKPDAISKAGEIIEIINKAGFTITKLKMMMLSRKEALDFHVDHQSRPFFNELIQFITTGPIIAMEILRDDAICEWKRLLGPANSGVARTDASESIRALFGTDGIRNAAHGPDSFASAAREMELFFPSSGGCGPANTAKFTNCTCCIVKPHAVSEGMLNTLYSVHFVNRRAMFIFLMYFMYRK

SEQ ID NO: 14 - DNA, 534 bp, Artificial Sequence
  NM23-H1 nucleotide sequence
atggtgctactgtctactttagggatcgtctttcaaggcgaggggcctcctatctcaagctgtgatacaggaaccatggccaactgtgagcgtaccttcattgcgatcaaaccagatggggtccagcggggtcttgtgggagagattatcaagcgttttgagcagaaaggattccgccttgttggtctgaaattcatgcaagcttccgaagatcttctcaaggaacactacgttgacctgaaggaccgtccattctttgccggcctggtgaaatacatgcactcagggccggtagttgccatggtctgggaggggctgaatgtggtgaagacgggccgagtcatgctcggggagaccaaccctgcagactccaagcctgggaccatccgtggagacttctgcatacaagttggcaggaacattatacatggcagtgattctgtggagagtgcagagaaggagatcggcttgtggtttcaccctgaggaactggtagattacacgagctgtgctcagaactggatctatgaatga

SEQ ID NO: 15 - protein, 177 aa, Artificial Sequence
  NM23-H1 describes amino acid sequence
MVLLSTLGIVFQGEGPPISSCDTGTMANCERTFIAIKPDGVQRGLVGEIIKRFEQKGFRLVGLKFMQASEDLLKEHYVDLKDRPFFAGLVKYMHSGPVVAMVWEGLNVVKTGRVMLGETNPADSKPGTIRGDFCIQVGRNIIHGSDSVESAEKEIGLWFHPEELVDYTSCAQNWIYE

SEQ ID NO: 16 - DNA, 534 bp, Artificial Sequence
  NM23-H1 S120G mutant nucleotide sequence
atggtgctactgtctactttagggatcgtctttcaaggcgaggggcctcctatctcaagctgtgatacaggaaccatggccaactgtgagcgtaccttcattgcgatcaaaccagatggggtccagcggggtcttgtgggagagattatcaagcgttttgagcagaaaggattccgccttgttggtctgaaattcatgcaagcttccgaagatcttctcaaggaacactacgttgacctgaaggaccgtccattctttgccggcctggtgaaatacatgcactcagggccggtagttgccatggtctgggaggggctgaatgtggtgaagacgggccgagtcatgctcggggagaccaaccctgcagactccaagcctgggaccatccgtggagacttctgcatacaagttggcaggaacattatacatggcggtgattctgtggagagtgcagagaaggagatcggcttgtggtttcaccctgaggaactggtagattacacgagctgtgctcagaactggatctatgaatga

SEQ ID NO: 17 - protein, 177 aa, Artificial Sequence
  NM23-H1 S120G mutant amino acid sequence
MVLLSTLGIVFQGEGPPISSCDTGTMANCERTFIAIKPDGVQRGLVGEIIKRFEQKGFRLVGLKFMQASEDLLKEHYVDLKDRPFFAGLVKYMHSGPVVAMVWEGLNVVKTGRVMLGETNPADSKPGTIRGDFCIQVGRNIIHGGDSVESAEKEIGLWFHPEELVDYTSCAQNWIYE

SEQ ID NO: 18 - DNA, 459 bp, Artificial Sequence
  NM23-H2 nucleotide sequence
atggccaacctggagcgcaccttcatcgccatcaagccggacggcgtgcagcgcggcctggtgggcgagatcatcaagcgcttcgagcagaagggattccgcctcgtggccatgaagttcctccgggcctctgaagaacacctgaagcagcactacattgacctgaaagaccgaccattcttccctgggctggtgaagtacatgaactcagggccggttgtggccatggtctgggaggggctgaacgtggtgaagacaggccgagtgatgcttggggagaccaatccagcagattcaaagccaggcaccattcgtggggacttctgcattcaggttggcaggaacatcattcatggcagtgattcagtaaaaagtgctgaaaaagaaatcagcctatggtttaagcctgaagaactggttgactacaagtcttgtgctcatgactgggtctatgaataa

SEQ ID NO: 19 - protein, 152 aa, Artificial Sequence
  NM23-H2 amino acid sequence
MANLERTFIAIKPDGVQRGLVGEIIKRFEQKGFRLVAMKFLRASEEHLKQHYIDLKDRPFFPGLVKYMNSGPVVAMVWEGLNVVKTGRVMLGETNPADSKPGTIRGDFCIQVGRNIIHGSDSVKSAEKEISLWFKPEELVDYKSCAHDWVYE

SEQ ID NO: 20 - DNA, 1023 bp, Artificial Sequence
  Human NM23-H7-2 sequence optimized for E. coli expression
atgcatgacgttaaaaatcaccgtacctttctgaaacgcacgaaatatgataatctgcatctggaagacctgtttattggcaacaaagtcaatgtgttctctcgtcagctggtgctgatcgattatggcgaccagtacaccgcgcgtcaactgggtagtcgcaaagaaaaaacgctggccctgattaaaccggatgcaatctccaaagctggcgaaattatcgaaattatcaacaaagcgggtttcaccatcacgaaactgaaaatgatgatgctgagccgtaaagaagccctggattttcatgtcgaccaccagtctcgcccgtttttcaatgaactgattcaattcatcaccacgggtccgattatcgcaatggaaattctgcgtgatgacgctatctgcgaatggaaacgcctgctgggcccggcaaactcaggtgttgcgcgtaccgatgccagtgaatccattcgcgctctgtttggcaccgatggtatccgtaatgcagcacatggtccggactcattcgcatcggcagctcgtgaaatggaactgtttttcccgagctctggcggttgcggtccggcaaacaccgccaaatttaccaattgtacgtgctgtattgtcaaaccgcacgcagtgtcagaaggcctgctgggtaaaattctgatggcaatccgtgatgctggctttgaaatctcggccatgcagatgttcaacatggaccgcgttaacgtcgaagaattctacgaagtttacaaaggcgtggttaccgaatatcacgatatggttacggaaatgtactccggtccgtgcgtcgcgatggaaattcagcaaaacaatgccaccaaaacgtttcgtgaattctgtggtccggcagatccggaaatcgcacgtcatctgcgtccgggtaccctgcgcgcaatttttggtaaaacgaaaatccagaacgctgtgcactgtaccgatctgccggaagacggtctgctggaagttcaatactttttcaaaattctggataattga

SEQ ID NO: 21 - protein, 340 aa, Artificial Sequence
  Human NM23-H7-2 sequence optimized for E. coli expression
MHDVKNHRTFLKRTKYDNLHLEDLFIGNKVNVFSRQLVLIDYGDQYTARQLGSRKEKTLALIKPDAISKAGEIIEIINKAGFTITKLKMMMLSRKEALDFHVDHQSRPFFNELIQFITTGPIIAMEILRDDAICEWKRLLGPANSGVARTDASESIRALFGTDGIRNAAHGPDSFASAAREMELFFPSSGGCGPANTAKFTNCTCCIVKPHAVSEGLLGKILMAIRDAGFEISAMQMFNMDRVNVEEFYEVYKGVVTEYHDMVTEMYSGPCVAMEIQQNNATKTFREFCGPADPEIARHLRPGTLRAIFGKTKIQNAVHCTDLPEDGLLEVQYFFKILDN

SEQ ID NO: 22 - DNA, 399 bp, Artificial Sequence
  Human NME7-A
atggaaaaaacgctagccctaattaaaccagatgcaatatcaaaggctggagaaataattgaaataataaacaaagctggatttactataaccaaactcaaaatgatgatgctttcaaggaaagaagcattggattttcatgtagatcaccagtcaagaccctttttcaatgagctgatccagtttattacaactggtcctattattgccatggagattttaagagatgatgctatatgtgaatggaaaagactgctgggacctgcaaactctggagtggcacgcacagatgcttctgaaagcattagagccctctttggaacagatggcataagaaatgcagcgcatggccctgattcttttgcttctgcggccagagaaatggagttgtttttttga

SEQ ID NO: 23 - protein, 132 aa, Artificial Sequence
  Human NME7-A
MEKTLALIKPDAISKAGEIIEIINKAGFTITKLKMMMLSRKEALDFHVDHQSRPFFNELIQFITTGPIIAMEILRDDAICEWKRLLGPANSGVARTDASESIRALFGTDGIRNAAHGPDSFASAAREMELFF

SEQ ID NO: 24 - DNA, 444 bp, Artificial Sequence
  Human NME7-A1
atggaaaaaacgctagccctaattaaaccagatgcaatatcaaaggctggagaaataattgaaataataaacaaagctggatttactataaccaaactcaaaatgatgatgctttcaaggaaagaagcattggattttcatgtagatcaccagtcaagaccctttttcaatgagctgatccagtttattacaactggtcctattattgccatggagattttaagagatgatgctatatgtgaatggaaaagactgctgggacctgcaaactctggagtggcacgcacagatgcttctgaaagcattagagccctctttggaacagatggcataagaaatgcagcgcatggccctgattcttttgcttctgcggccagagaaatggagttgttttttccttcaagtggaggttgtgggccggcaaacactgctaaatttacttga

SEQ ID NO: 25 - protein, 147 aa, Artificial Sequence
  Human NME7-A1
MEKTLALIKPDAISKAGEIIEIINKAGFTITKLKMMMLSRKEALDFHVDHQSRPFFNELIQFITTGPIIAMEILRDDAICEWKRLLGPANSGVARTDASESIRALFGTDGIRNAAHGPDSFASAAREMELFFPSSGGCGPANTAKFT

SEQ ID NO: 26 - DNA, 669 bp, Artificial Sequence
  Human NME7-A2
atgaatcatagtgaaagattcgttttcattgcagagtggtatgatccaaatgcttcacttcttcgacgttatgagcttttattttacccaggggatggatctgttgaaatgcatgatgtaaagaatcatcgcacctttttaaagcggaccaaatatgataacctgcacttggaagatttatttataggcaacaaagtgaatgtcttttctcgacaactggtattaattgactatggggatcaatatacagctcgccagctgggcagtaggaaagaaaaaacgctagccctaattaaaccagatgcaatatcaaaggctggagaaataattgaaataataaacaaagctggatttactataaccaaactcaaaatgatgatgctttcaaggaaagaagcattggattttcatgtagatcaccagtcaagaccctttttcaatgagctgatccagtttattacaactggtcctattattgccatggagattttaagagatgatgctatatgtgaatggaaaagactgctgggacctgcaaactctggagtggcacgcacagatgcttctgaaagcattagagccctctttggaacagatggcataagaaatgcagcgcatggccctgattcttttgcttctgcggccagagaaatggagttgtttttttga

SEQ ID NO: 27 - protein, 222 aa, Artificial Sequence
  Human NME7-A2
MNHSERFVFIAEWYDPNASLLRRYELLFYPGDGSVEMHDVKNHRTFLKRTKYDNLHLEDLFIGNKVNVFSRQLVLIDYGDQYTARQLGSRKEKTLALIKPDAISKAGEIIEIINKAGFTITKLKMMMLSRKEALDFHVDHQSRPFFNELIQFITTGPIIAMEILRDDAICEWKRLLGPANSGVARTDASESIRALFGTDGIRNAAHGPDSFASAAREMELFF

SEQ ID NO: 28 - DNA, 714 bp, Artificial Sequence
  Human NME7-A3
atgaatcatagtgaaagattcgttttcattgcagagtggtatgatccaaatgcttcacttcttcgacgttatgagcttttattttacccaggggatggatctgttgaaatgcatgatgtaaagaatcatcgcacctttttaaagcggaccaaatatgataacctgcacttggaagatttatttataggcaacaaagtgaatgtcttttctcgacaactggtattaattgactatggggatcaatatacagctcgccagctgggcagtaggaaagaaaaaacgctagccctaattaaaccagatgcaatatcaaaggctggagaaataattgaaataataaacaaagctggatttactataaccaaactcaaaatgatgatgctttcaaggaaagaagcattggattttcatgtagatcaccagtcaagaccctttttcaatgagctgatccagtttattacaactggtcctattattgccatggagattttaagagatgatgctatatgtgaatggaaaagactgctgggacctgcaaactctggagtggcacgcacagatgcttctgaaagcattagagccctctttggaacagatggcataagaaatgcagcgcatggccctgattcttttgcttctgcggccagagaaatggagttgttttttccttcaagtggaggttgtgggccggcaaacactgctaaatttacttga

SEQ ID NO: 29 - protein, 237 aa, Artificial Sequence
  Human NME7-A3
MNHSERFVFIAEWYDPNASLLRRYELLFYPGDGSVEMHDVKNHRTFLKRTKYDNLHLEDLFIGNKVNVFSRQLVLIDYGDQYTARQLGSRKEKTLALIKPDAISKAGEIIEIINKAGFTITKLKMMMLSRKEALDFHVDHQSRPFFNELIQFITTGPIIAMEILRDDAICEWKRLLGPANSGVARTDASESIRALFGTDGIRNAAHGPDSFASAAREMELFFPSSGGCGPANTAKFT

SEQ ID NO: 30 - DNA, 408 bp, Artificial Sequence
  Human NME7-B
atgaattgtacctgttgcattgttaaaccccatgctgtcagtgaaggactgttgggaaagatcctgatggctatccgagatgcaggttttgaaatctcagctatgcagatgttcaatatggatcgggttaatgttgaggaattctatgaagtttataaaggagtagtgaccgaatatcatgacatggtgacagaaatgtattctggcccttgtgtagcaatggagattcaacagaataatgctacaaagacatttcgagaattttgtggacctgctgatcctgaaattgcccggcatttacgccctggaactctcagagcaatctttggtaaaactaagatccagaatgctgttcactgtactgatctgccagaggatggcctattagaggttcaatacttcttctga

SEQ ID NO: 31 - protein, 135 aa, Artificial Sequence
  Human NME7-B
MNCTCCIVKPHAVSEGLLGKILMAIRDAGFEISAMQMFNMDRVNVEEFYEVYKGVVTEYHDMVTEMYSGPCVAMEIQQNNATKTFREFCGPADPEIARHLRPGTLRAIFGKTKIQNAVHCTDLPEDGLLEVQYFF

SEQ ID NO: 32 - DNA, 426 bp, Artificial Sequence
  Human NME7-B1
atgaattgtacctgttgcattgttaaaccccatgctgtcagtgaaggactgttgggaaagatcctgatggctatccgagatgcaggttttgaaatctcagctatgcagatgttcaatatggatcgggttaatgttgaggaattctatgaagtttataaaggagtagtgaccgaatatcatgacatggtgacagaaatgtattctggcccttgtgtagcaatggagattcaacagaataatgctacaaagacatttcgagaattttgtggacctgctgatcctgaaattgcccggcatttacgccctggaactctcagagcaatctttggtaaaactaagatccagaatgctgttcactgtactgatctgccagaggatggcctattagaggttcaatacttcttcaagatcttggataattagtga

SEQ ID NO: 33 - protein, 140 aa, Artificial Sequence
  Human NME7-B1
MNCTCCIVKPHAVSEGLLGKILMAIRDAGFEISAMQMFNMDRVNVEEFYEVYKGVVTEYHDMVTEMYSGPCVAMEIQQNNATKTFREFCGPADPEIARHLRPGTLRAIFGKTKIQNAVHCTDLPEDGLLEVQYFFKILDN

SEQ ID NO: 34 - DNA, 453 bp, Artificial Sequence
  Human NME7-B2
atgccttcaagtggaggttgtgggccggcaaacactgctaaatttactaattgtacctgttgcattgttaaaccccatgctgtcagtgaaggactgttgggaaagatcctgatggctatccgagatgcaggttttgaaatctcagctatgcagatgttcaatatggatcgggttaatgttgaggaattctatgaagtttataaaggagtagtgaccgaatatcatgacatggtgacagaaatgtattctggcccttgtgtagcaatggagattcaacagaataatgctacaaagacatttcgagaattttgtggacctgctgatcctgaaattgcccggcatttacgccctggaactctcagagcaatctttggtaaaactaagatccagaatgctgttcactgtactgatctgccagaggatggcctattagaggttcaatacttcttctga

SEQ ID NO: 35 - protein, 150 aa, Artificial Sequence
  Human NME7-B2
MPSSGGCGPANTAKFTNCTCCIVKPHAVSEGLLGKILMAIRDAGFEISAMQMFNMDRVNVEEFYEVYKGVVTEYHDMVTEMYSGPCVAMEIQQNNATKTFREFCGPADPEIARHLRPGTLRAIFGKTKIQNAVHCTDLPEDGLLEVQYFF

SEQ ID NO: 36 - DNA, 471 bp, Artificial Sequence
  Human NME7-B3
atgccttcaagtggaggttgtgggccggcaaacactgctaaatttactaattgtacctgttgcattgttaaaccccatgctgtcagtgaaggactgttgggaaagatcctgatggctatccgagatgcaggttttgaaatctcagctatgcagatgttcaatatggatcgggttaatgttgaggaattctatgaagtttataaaggagtagtgaccgaatatcatgacatggtgacagaaatgtattctggcccttgtgtagcaatggagattcaacagaataatgctacaaagacatttcgagaattttgtggacctgctgatcctgaaattgcccggcatttacgccctggaactctcagagcaatctttggtaaaactaagatccagaatgctgttcactgtactgatctgccagaggatggcctattagaggttcaatacttcttcaagatcttggataattagtga

SEQ ID NO: 37 - protein, 155 aa, Artificial Sequence
  Human NME7-B3
MPSSGGCGPANTAKFTNCTCCIVKPHAVSEGLLGKILMAIRDAGFEISAMQMFNMDRVNVEEFYEVYKGVVTEYHDMVTEMYSGPCVAMEIQQNNATKTFREFCGPADPEIARHLRPGTLRAIFGKTKIQNAVHCTDLPEDGLLEVQYFFKILDN

SEQ ID NO: 38 - DNA, 864 bp, Artificial Sequence
  Human NME7-AB
atggaaaaaacgctagccctaattaaaccagatgcaatatcaaaggctggagaaataattgaaataataaacaaagctggatttactataaccaaactcaaaatgatgatgctttcaaggaaagaagcattggattttcatgtagatcaccagtcaagaccctttttcaatgagctgatccagtttattacaactggtcctattattgccatggagattttaagagatgatgctatatgtgaatggaaaagactgctgggacctgcaaactctggagtggcacgcacagatgcttctgaaagcattagagccctctttggaacagatggcataagaaatgcagcgcatggccctgattcttttgcttctgcggccagagaaatggagttgttttttccttcaagtggaggttgtgggccggcaaacactgctaaatttactaattgtacctgttgcattgttaaaccccatgctgtcagtgaaggactgttgggaaagatcctgatggctatccgagatgcaggttttgaaatctcagctatgcagatgttcaatatggatcgggttaatgttgaggaattctatgaagtttataaaggagtagtgaccgaatatcatgacatggtgacagaaatgtattctggcccttgtgtagcaatggagattcaacagaataatgctacaaagacatttcgagaattttgtggacctgctgatcctgaaattgcccggcatttacgccctggaactctcagagcaatctttggtaaaactaagatccagaatgctgttcactgtactgatctgccagaggatggcctattagaggttcaatacttcttcaagatcttggataattagtga

SEQ ID NO: 39 - protein, 286 aa, Artificial Sequence
  Human NME7-AB
MEKTLALIKPDAISKAGEIIEIINKAGFTITKLKMMMLSRKEALDFHVDHQSRPFFNELIQFITTGPIIAMEILRDDAICEWKRLLGPANSGVARTDASESIRALFGTDGIRNAAHGPDSFASAAREMELFFPSSGGCGPANTAKFTNCTCCIVKPHAVSEGLLGKILMAIRDAGFEISAMQMFNMDRVNVEEFYEVYKGVVTEYHDMVTEMYSGPCVAMEIQQNNATKTFREFCGPADPEIARHLRPGTLRAIFGKTKIQNAVHCTDLPEDGLLEVQYFFKILDN

SEQ ID NO: 40 - DNA, 846 bp, Artificial Sequence
  Human NME7-AB1
atggaaaaaacgctagccctaattaaaccagatgcaatatcaaaggctggagaaataattgaaataataaacaaagctggatttactataaccaaactcaaaatgatgatgctttcaaggaaagaagcattggattttcatgtagatcaccagtcaagaccctttttcaatgagctgatccagtttattacaactggtcctattattgccatggagattttaagagatgatgctatatgtgaatggaaaagactgctgggacctgcaaactctggagtggcacgcacagatgcttctgaaagcattagagccctctttggaacagatggcataagaaatgcagcgcatggccctgattcttttgcttctgcggccagagaaatggagttgttttttccttcaagtggaggttgtgggccggcaaacactgctaaatttactaattgtacctgttgcattgttaaaccccatgctgtcagtgaaggactgttgggaaagatcctgatggctatccgagatgcaggttttgaaatctcagctatgcagatgttcaatatggatcgggttaatgttgaggaattctatgaagtttataaaggagtagtgaccgaatatcatgacatggtgacagaaatgtattctggcccttgtgtagcaatggagattcaacagaataatgctacaaagacatttcgagaattttgtggacctgctgatcctgaaattgcccggcatttacgccctggaactctcagagcaatctttggtaaaactaagatccagaatgctgttcactgtactgatctgccagaggatggcctattagaggttcaatacttcttctga

SEQ ID NO: 41 - protein, 281 aa, Artificial Sequence
  Human NME7-AB1
MEKTLALIKPDAISKAGEIIEIINKAGFTITKLKMMMLSRKEALDFHVDHQSRPFFNELIQFITTGPIIAMEILRDDAICEWKRLLGPANSGVARTDASESIRALFGTDGIRNAAHGPDSFASAAREMELFFPSSGGCGPANTAKFTNCTCCIVKPHAVSEGLLGKILMAIRDAGFEISAMQMFNMDRVNVEEFYEVYKGVVTEYHDMVTEMYSGPCVAMEIQQNNATKTFREFCGPADPEIARHLRPGTLRAIFGKTKIQNAVHCTDLPEDGLLEVQYFF

SEQ ID NO: 42 - DNA, 399 bp, Artificial Sequence
  Human NME7-A sequence optimized for E. coli expression
atggaaaaaacgctggccctgattaaaccggatgcaatctccaaagctggcgaaattatcgaaattatcaacaaagcgggtttcaccatcacgaaactgaaaatgatgatgctgagccgtaaagaagccctggattttcatgtcgaccaccagtctcgcccgtttttcaatgaactgattcaattcatcaccacgggtccgattatcgcaatggaaattctgcgtgatgacgctatctgcgaatggaaacgcctgctgggcccggcaaactcaggtgttgcgcgtaccgatgccagtgaatccattcgcgctctgtttggcaccgatggtatccgtaatgcagcacatggtccggactcattcgcatcggcagctcgtgaaatggaactgtttttctga

SEQ ID NO: 43 - protein, 132 aa, Artificial Sequence; identical to SEQ ID NO: 23
  Human NME7-A sequence optimized for E. coli expression

SEQ ID NO: 44 - DNA, 444 bp, Artificial Sequence
  Human NME7-A1 sequence optimized for E. coli expression
atggaaaaaacgctggccctgattaaaccggatgcaatctccaaagctggcgaaattatcgaaattatcaacaaagcgggtttcaccatcacgaaactgaaaatgatgatgctgagccgtaaagaagccctggattttcatgtcgaccaccagtctcgcccgtttttcaatgaactgattcaattcatcaccacgggtccgattatcgcaatggaaattctgcgtgatgacgctatctgcgaatggaaacgcctgctgggcccggcaaactcaggtgttgcgcgtaccgatgccagtgaatccattcgcgctctgtttggcaccgatggtatccgtaatgcagcacatggtccggactcattcgcatcggcagctcgtgaaatggaactgtttttcccgagctctggcggttgcggtccggcaaacaccgccaaatttacctga

SEQ ID NO: 45 - protein, 147 aa, Artificial Sequence; identical to SEQ ID NO: 25
  Human NME7-A1 sequence optimized for E. coli expression

SEQ ID NO: 46 - DNA, 669 bp, Artificial Sequence
  Human NME7-A2 sequence optimized for E. coli expression
atgaatcactccgaacgctttgtttttatcgccgaatggtatgacccgaatgcttccctgctgcgccgctacgaactgctgttttatccgggcgatggtagcgtggaaatgcatgacgttaaaaatcaccgtacctttctgaaacgcacgaaatatgataatctgcatctggaagacctgtttattggcaacaaagtcaatgtgttctctcgtcagctggtgctgatcgattatggcgaccagtacaccgcgcgtcaactgggtagtcgcaaagaaaaaacgctggccctgattaaaccggatgcaatctccaaagctggcgaaattatcgaaattatcaacaaagcgggtttcaccatcacgaaactgaaaatgatgatgctgagccgtaaagaagccctggattttcatgtcgaccaccagtctcgcccgtttttcaatgaactgattcaattcatcaccacgggtccgattatcgcaatggaaattctgcgtgatgacgctatctgcgaatggaaacgcctgctgggcccggcaaactcaggtgttgcgcgtaccgatgccagtgaatccattcgcgctctgtttggcaccgatggtatccgtaatgcagcacatggtccggactcattcgcatcggcagctcgtgaaatggaactgtttttctga

SEQ ID NO: 47 - protein, 222 aa, Artificial Sequence; identical to SEQ ID NO: 27
  Human NME7-A2 sequence optimized for E. coli expression

SEQ ID NO: 48 - DNA, 714 bp, Artificial Sequence
  Human NME7-A3 sequence optimized for E. coli expression
atgaatcactccgaacgctttgtttttatcgccgaatggtatgacccgaatgcttccctgctgcgccgctacgaactgctgttttatccgggcgatggtagcgtggaaatgcatgacgttaaaaatcaccgtacctttctgaaacgcacgaaatatgataatctgcatctggaagacctgtttattggcaacaaagtcaatgtgttctctcgtcagctggtgctgatcgattatggcgaccagtacaccgcgcgtcaactgggtagtcgcaaagaaaaaacgctggccctgattaaaccggatgcaatctccaaagctggcgaaattatcgaaattatcaacaaagcgggtttcaccatcacgaaactgaaaatgatgatgctgagccgtaaagaagccctggattttcatgtcgaccaccagtctcgcccgtttttcaatgaactgattcaattcatcaccacgggtccgattatcgcaatggaaattctgcgtgatgacgctatctgcgaatggaaacgcctgctgggcccggcaaactcaggtgttgcgcgtaccgatgccagtgaatccattcgcgctctgtttggcaccgatggtatccgtaatgcagcacatggtccggactcattcgcatcggcagctcgtgaaatggaactgtttttcccgagctctggcggttgcggtccggcaaacaccgccaaatttacctga

SEQ ID NO: 49 - protein, 237 aa, Artificial Sequence; identical to SEQ ID NO: 29
  Human NME7-A3 sequence optimized for E. coli expression

SEQ ID NO: 50 - DNA, 408 bp, Artificial Sequence
  Human NME7-B sequence optimized for E. coli expression
atgaattgtacgtgctgtattgtcaaaccgcacgcagtgtcagaaggcctgctgggtaaaattctgatggcaatccgtgatgctggctttgaaatctcggccatgcagatgttcaacatggaccgcgttaacgtcgaagaattctacgaagtttacaaaggcgtggttaccgaatatcacgatatggttacggaaatgtactccggtccgtgcgtcgcgatggaaattcagcaaaacaatgccaccaaaacgtttcgtgaattctgtggtccggcagatccggaaatcgcacgtcatctgcgtccgggtaccctgcgcgcaatttttggtaaaacgaaaatccagaacgctgtgcactgtaccgatctgccggaagacggtctgctggaagttcaatactttttctga

SEQ ID NO: 51 - protein, 135 aa, Artificial Sequence; identical to SEQ ID NO: 31
  Human NME7-B sequence optimized for E. coli expression

SEQ ID NO: 52 - DNA, 423 bp, Artificial Sequence
  Human NME7-B1 sequence optimized for E. coli expression
atgaattgtacgtgctgtattgtcaaaccgcacgcagtgtcagaaggcctgctgggtaaaattctgatggcaatccgtgatgctggctttgaaatctcggccatgcagatgttcaacatggaccgcgttaacgtcgaagaattctacgaagtttacaaaggcgtggttaccgaatatcacgatatggttacggaaatgtactccggtccgtgcgtcgcgatggaaattcagcaaaacaatgccaccaaaacgtttcgtgaattctgtggtccggcagatccggaaatcgcacgtcatctgcgtccgggtaccctgcgcgcaatttttggtaaaacgaaaatccagaacgctgtgcactgtaccgatctgccggaagacggtctgctggaagttcaatactttttcaaaattctggataattga

SEQ ID NO: 53 - protein, 140 aa, Artificial Sequence; identical to SEQ ID NO: 33
  Human NME7-B1 sequence optimized for E. coli expression

SEQ ID NO: 54 - DNA, 453 bp, Artificial Sequence
  human NME7-B2 sequence optimized for E. coli expression
atgccgagctctggcggttgcggtccggcaaacaccgccaaatttaccaattgtacgtgctgtattgtcaaaccgcacgcagtgtcagaaggcctgctgggtaaaattctgatggcaatccgtgatgctggctttgaaatctcggccatgcagatgttcaacatggaccgcgttaacgtcgaagaattctacgaagtttacaaaggcgtggttaccgaatatcacgatatggttacggaaatgtactccggtccgtgcgtcgcgatggaaattcagcaaaacaatgccaccaaaacgtttcgtgaattctgtggtccggcagatccggaaatcgcacgtcatctgcgtccgggtaccctgcgcgcaatttttggtaaaacgaaaatccagaacgctgtgcactgtaccgatctgccggaagacggtctgctggaagttcaatactttttctga

SEQ ID NO: 55 - protein, 150 aa, Artificial Sequence; identical to SEQ ID NO: 35
  human NME7-B2 sequence optimized for E. coli expression

SEQ ID NO: 56 - DNA, 468 bp, Artificial Sequence
  Human NME7-B3 sequence optimized for E. coli expression
atgccgagctctggcggttgcggtccggcaaacaccgccaaatttaccaattgtacgtgctgtattgtcaaaccgcacgcagtgtcagaaggcctgctgggtaaaattctgatggcaatccgtgatgctggctttgaaatctcggccatgcagatgttcaacatggaccgcgttaacgtcgaagaattctacgaagtttacaaaggcgtggttaccgaatatcacgatatggttacggaaatgtactccggtccgtgcgtcgcgatggaaattcagcaaaacaatgccaccaaaacgtttcgtgaattctgtggtccggcagatccggaaatcgcacgtcatctgcgtccgggtaccctgcgcgcaatttttggtaaaacgaaaatccagaacgctgtgcactgtaccgatctgccggaagacggtctgctggaagttcaatactttttcaaaattctggataattga

SEQ ID NO: 57 - protein, 155 aa, Artificial Sequence; identical to SEQ ID NO: 37
  Human NME7-B3 sequence optimized for E. coli expression

SEQ ID NO: 58 - DNA, 861 bp, Artificial Sequence
  Human NME7-AB sequence optimized for E. coli expression
atggaaaaaacgctggccctgattaaaccggatgcaatctccaaagctggcgaaattatcgaaattatcaacaaagcgggtttcaccatcacgaaactgaaaatgatgatgctgagccgtaaagaagccctggattttcatgtcgaccaccagtctcgcccgtttttcaatgaactgattcaattcatcaccacgggtccgattatcgcaatggaaattctgcgtgatgacgctatctgcgaatggaaacgcctgctgggcccggcaaactcaggtgttgcgcgtaccgatgccagtgaatccattcgcgctctgtttggcaccgatggtatccgtaatgcagcacatggtccggactcattcgcatcggcagctcgtgaaatggaactgtttttcccgagctctggcggttgcggtccggcaaacaccgccaaatttaccaattgtacgtgctgtattgtcaaaccgcacgcagtgtcagaaggcctgctgggtaaaattctgatggcaatccgtgatgctggctttgaaatctcggccatgcagatgttcaacatggaccgcgttaacgtcgaagaattctacgaagtttacaaaggcgtggttaccgaatatcacgatatggttacggaaatgtactccggtccgtgcgtcgcgatggaaattcagcaaaacaatgccaccaaaacgtttcgtgaattctgtggtccggcagatccggaaatcgcacgtcatctgcgtccgggtaccctgcgcgcaatttttggtaaaacgaaaatccagaacgctgtgcactgtaccgatctgccggaagacggtctgctggaagttcaatactttttcaaaattctggataattga

SEQ ID NO: 59 - protein, 286 aa, Artificial Sequence; identical to SEQ ID NO: 39
  Human NME7-AB sequence optimized for E. coli expression

SEQ ID NO: 60 - DNA, 846 bp, Artificial Sequence
  Human NME7-AB1 sequence optimized for E. coli expression
atggaaaaaacgctggccctgattaaaccggatgcaatctccaaagctggcgaaattatcgaaattatcaacaaagcgggtttcaccatcacgaaactgaaaatgatgatgctgagccgtaaagaagccctggattttcatgtcgaccaccagtctcgcccgtttttcaatgaactgattcaattcatcaccacgggtccgattatcgcaatggaaattctgcgtgatgacgctatctgcgaatggaaacgcctgctgggcccggcaaactcaggtgttgcgcgtaccgatgccagtgaatccattcgcgctctgtttggcaccgatggtatccgtaatgcagcacatggtccggactcattcgcatcggcagctcgtgaaatggaactgtttttcccgagctctggcggttgcggtccggcaaacaccgccaaatttaccaattgtacgtgctgtattgtcaaaccgcacgcagtgtcagaaggcctgctgggtaaaattctgatggcaatccgtgatgctggctttgaaatctcggccatgcagatgttcaacatggaccgcgttaacgtcgaagaattctacgaagtttacaaaggcgtggttaccgaatatcacgatatggttacggaaatgtactccggtccgtgcgtcgcgatggaaattcagcaaaacaatgccaccaaaacgtttcgtgaattctgtggtccggcagatccggaaatcgcacgtcatctgcgtccgggtaccctgcgcgcaatttttggtaaaacgaaaatccagaacgctgtgcactgtaccgatctgccggaagacggtctgctggaagttcaatactttttctga

SEQ ID NO: 61 - protein, 281 aa, Artificial Sequence; identical to SEQ ID NO: 41
  Human NME7-AB1 sequence optimized for E. coli expression

SEQ ID NO: 62 - DNA, 570 bp, Artificial Sequence
  Mouse NME6
atgacctccatcttgcgaagtccccaagctcttcagctcacactagccctgatcaagcctgatgcagttgcccacccactgatcctggaggctgttcatcagcagattctgagcaacaagttcctcattgtacgaacgagggaactgcagtggaagctggaggactgccggaggttttaccgagagcatgaagggcgttttttctatcagcggctggtggagttcatgacaagtgggccaatccgagcctatatccttgcccacaaagatgccatccaactttggaggacactgatgggacccaccagagtatttcgagcacgctatatagccccagattcaattcgtggaagtttgggcctcactgacacccgaaatactacccatggctcagactccgtggtttccgccagcagagagattgcagccttcttccctgacttcagtgaacagcgctggtatgaggaggaggaaccccagctgcggtgtggtcctgtgcactacagtccagaggaaggtatccactgtgcagctgaaacaggaggccacaaacaacctaacaaaacctag

SEQ ID NO: 63 - protein, 189 aa, Artificial Sequence
  Mouse NME6
MTSILRSPQALQLTLALIKPDAVAHPLILEAVHQQILSNKFLIVRTRELQWKLEDCRRFYREHEGRFFYQRLVEFMTSGPIRAYILAHKDAIQLWRTLMGPTRVFRARYIAPDSIRGSLGLTDTRNTTHGSDSVVSASREIAAFFPDFSEQRWYEEEEPQLRCGPVHYSPEEGIHCAAETGGHKQPNKT

SEQ ID NO: 64 - DNA, 585 bp, Artificial Sequence
  Human NME6
atgacccagaatctggggagtgagatggcctcaatcttgcgaagccctcaggctctccagctcactctagccctgatcaagcctgacgcagtcgcccatccactgattctggaggctgttcatcagcagattctaagcaacaagttcctgattgtacgaatgagagaactactgtggagaaaggaagattgccagaggttttaccgagagcatgaagggcgttttttctatcagaggctggtggagttcatggccagcgggccaatccgagcctacatccttgcccacaaggatgccatccagctctggaggacgctcatgggacccaccagagtgttccgagcacgccatgtggccccagattctatccgtgggagtttcggcctcactgacacccgcaacaccacccatggttcggactctgtggtttcagccagcagagagattgcagccttcttccctgacttcagtgaacagcgctggtatgaggaggaagagccccagttgcgctgtggccctgtgtgctatagcccagagggaggtgtccactatgtagctggaacaggaggcctaggaccagcctga

SEQ ID NO: 65 - protein, 194 aa, Artificial Sequence
  Human NME6
MTQNLGSEMASILRSPQALQLTLALIKPDAVAHPLILEAVHQQILSNKFLIVRMRELLWRKEDCQRFYREHEGRFFYQRLVEFMASGPIRAYILAHKDAIQLWRTLMGPTRVFRARHVAPDSIRGSFGLTDTRNTTHGSDSVVSASREIAAFFPDFSEQRWYEEEEPQLRCGPVCYSPEGGVHYVAGTGGLGPA

SEQ ID NO: 66 - DNA, 525 bp, Artificial Sequence
  Human NME6 1
atgacccagaatctggggagtgagatggcctcaatcttgcgaagccctcaggctctccagctcactctagccctgatcaagcctgacgcagtcgcccatccactgattctggaggctgttcatcagcagattctaagcaacaagttcctgattgtacgaatgagagaactactgtggagaaaggaagattgccagaggttttaccgagagcatgaagggcgttttttctatcagaggctggtggagttcatggccagcgggccaatccgagcctacatccttgcccacaaggatgccatccagctctggaggacgctcatgggacccaccagagtgttccgagcacgccatgtggccccagattctatccgtgggagtttcggcctcactgacacccgcaacaccacccatggttcggactctgtggtttcagccagcagagagattgcagccttcttccctgacttcagtgaacagcgctggtatgaggaggaagagccccagttgcgctgtggccctgtgtga

SEQ ID NO: 67 - protein, 174 aa, Artificial Sequence
  Human NME6 1
MTQNLGSEMASILRSPQALQLTLALIKPDAVAHPLILEAVHQQILSNKFLIVRMRELLWRKEDCQRFYREHEGRFFYQRLVEFMASGPIRAYILAHKDAIQLWRTLMGPTRVFRARHVAPDSIRGSFGLTDTRNTTHGSDSVVSASREIAAFFPDFSEQRWYEEEEPQLRCGPV

SEQ ID NO: 68 - DNA, 468 bp, Artificial Sequence
  Human NME6 2
atgctcactctagccctgatcaagcctgacgcagtcgcccatccactgattctggaggctgttcatcagcagattctaagcaacaagttcctgattgtacgaatgagagaactactgtggagaaaggaagattgccagaggttttaccgagagcatgaagggcgttttttctatcagaggctggtggagttcatggccagcgggccaatccgagcctacatccttgcccacaaggatgccatccagctctggaggacgctcatgggacccaccagagtgttccgagcacgccatgtggccccagattctatccgtgggagtttcggcctcactgacacccgcaacaccacccatggttcggactctgtggtttcagccagcagagagattgcagccttcttccctgacttcagtgaacagcgctggtatgaggaggaagagccccagttgcgctgtggccctgtgtga

SEQ ID NO: 69 - protein, 155 aa, Artificial Sequence
  Human NME6 2
MLTLALIKPDAVAHPLILEAVHQQILSNKFLIVRMRELLWRKEDCQRFYREHEGRFFYQRLVEFMASGPIRAYILAHKDAIQLWRTLMGPTRVFRARHVAPDSIRGSFGLTDTRNTTHGSDSVVSASREIAAFFPDFSEQRWYEEEEPQLRCGPV

SEQ ID NO: 70 - DNA, 528 bp, Artificial Sequence
  Human NME6 3
atgctcactctagccctgatcaagcctgacgcagtcgcccatccactgattctggaggctgttcatcagcagattctaagcaacaagttcctgattgtacgaatgagagaactactgtggagaaaggaagattgccagaggttttaccgagagcatgaagggcgttttttctatcagaggctggtggagttcatggccagcgggccaatccgagcctacatccttgcccacaaggatgccatccagctctggaggacgctcatgggacccaccagagtgttccgagcacgccatgtggccccagattctatccgtgggagtttcggcctcactgacacccgcaacaccacccatggttcggactctgtggtttcagccagcagagagattgcagccttcttccctgacttcagtgaacagcgctggtatgaggaggaagagccccagttgcgctgtggccctgtgtgctatagcccagagggaggtgtccactatgtagctggaacaggaggcctaggaccagcctga

SEQ ID NO: 71 - protein, 175 aa, Artificial Sequence
  Human NME6 3
MLTLALIKPDAVAHPLILEAVHQQILSNKFLIVRMRELLWRKEDCQRFYREHEGRFFYQRLVEFMASGPIRAYILAHKDAIQLWRTLMGPTRVFRARHVAPDSIRGSFGLTDTRNTTHGSDSVVSASREIAAFFPDFSEQRWYEEEEPQLRCGPVCYSPEGGVHYVAGTGGLGPA

SEQ ID NO: 72 - DNA, 585 bp, Artificial Sequence
  Human NME6 sequence optimized for E. coli expression
atgacgcaaaatctgggctcggaaatggcaagtatcctgcgctccccgcaagcactgcaactgaccctggctctgatcaaaccggacgctgttgctcatccgctgattctggaagcggtccaccagcaaattctgagcaacaaatttctgatcgtgcgtatgcgcgaactgctgtggcgtaaagaagattgccagcgtttttatcgcgaacatgaaggccgtttcttttatcaacgcctggttgaattcatggcctctggtccgattcgcgcatatatcctggctcacaaagatgcgattcagctgtggcgtaccctgatgggtccgacgcgcgtctttcgtgcacgtcatgtggcaccggactcaatccgtggctcgttcggtctgaccgatacgcgcaataccacgcacggtagcgactctgttgttagtgcgtcccgtgaaatcgcggcctttttcccggacttctccgaacagcgttggtacgaagaagaagaaccgcaactgcgctgtggcccggtctgttattctccggaaggtggtgtccattatgtggcgggcacgggtggtctgggtccggcatga

SEQ ID NO: 73 - protein, 194 aa, Artificial Sequence; identical to SEQ ID NO: 65
  Human NME6 sequence optimized for E. coli expression

SEQ ID NO: 74 - DNA, 525 bp, Artificial Sequence
  Human NME6 1 sequence optimized for E. coli expression
atgacgcaaaatctgggctcggaaatggcaagtatcctgcgctccccgcaagcactgcaactgaccctggctctgatcaaaccggacgctgttgctcatccgctgattctggaagcggtccaccagcaaattctgagcaacaaatttctgatcgtgcgtatgcgcgaactgctgtggcgtaaagaagattgccagcgtttttatcgcgaacatgaaggccgtttcttttatcaacgcctggttgaattcatggcctctggtccgattcgcgcatatatcctggctcacaaagatgcgattcagctgtggcgtaccctgatgggtccgacgcgcgtctttcgtgcacgtcatgtggcaccggactcaatccgtggctcgttcggtctgaccgatacgcgcaataccacgcacggtagcgactctgttgttagtgcgtcccgtgaaatcgcggcctttttcccggacttctccgaacagcgttggtacgaagaagaagaaccgcaactgcgctgtggcccggtctga

SEQ ID NO: 75 - protein, 174 aa, Artificial Sequence; identical to SEQ ID NO: 67
  Human NME6 1 sequence optimized for E. coli expression

SEQ ID NO: 76 - DNA, 468 bp, Artificial Sequence
  Human NME6 2 sequence optimized for E. coli expression
atgctgaccctggctctgatcaaaccggacgctgttgctcatccgctgattctggaagcggtccaccagcaaattctgagcaacaaatttctgatcgtgcgtatgcgcgaactgctgtggcgtaaagaagattgccagcgtttttatcgcgaacatgaaggccgtttcttttatcaacgcctggttgaattcatggcctctggtccgattcgcgcatatatcctggctcacaaagatgcgattcagctgtggcgtaccctgatgggtccgacgcgcgtctttcgtgcacgtcatgtggcaccggactcaatccgtggctcgttcggtctgaccgatacgcgcaataccacgcacggtagcgactctgttgttagtgcgtcccgtgaaatcgcggcctttttcccggacttctccgaacagcgttggtacgaagaagaagaaccgcaactgcgctgtggcccggtctga

SEQ ID NO: 77 - protein, 155 aa, Artificial Sequence; identical to SEQ ID NO: 69
  Human NME6 2 sequence optimized for E. coli expression

SEQ ID NO: 78 - DNA, 528 bp, Artificial Sequence
  Human NME6 3 sequence optimized for E. coli expression
atgctgaccctggctctgatcaaaccggacgctgttgctcatccgctgattctggaagcggtccaccagcaaattctgagcaacaaatttctgatcgtgcgtatgcgcgaactgctgtggcgtaaagaagattgccagcgtttttatcgcgaacatgaaggccgtttcttttatcaacgcctggttgaattcatggcctctggtccgattcgcgcatatatcctggctcacaaagatgcgattcagctgtggcgtaccctgatgggtccgacgcgcgtctttcgtgcacgtcatgtggcaccggactcaatccgtggctcgttcggtctgaccgatacgcgcaataccacgcacggtagcgactctgttgttagtgcgtcccgtgaaatcgcggcctttttcccggacttctccgaacagcgttggtacgaagaagaagaaccgcaactgcgctgtggcccggtctgttattctccggaaggtggtgtccattatgtggcgggcacgggtggtctgggtccggcatga

SEQ ID NO: 79 - protein, 175 aa, Artificial Sequence; identical to SEQ ID NO: 71
  Human NME6 3 sequence optimized for E. coli expression

SEQ ID NO: 80 - DNA, 1306 bp, Artificial Sequence
  OriGene-NME7-1 full length
gacgttgtatacgactcctatagggcggccgggaattcgtcgactggatccggtaccgaggagatctgccgccgcgatcgccatgaatcatagtgaaagattcgttttcattgcagagtggtatgatccaaatgcttcacttcttcgacgttatgagcttttattttacccaggggatggatctgttgaaatgcatgatgtaaagaatcatcgcacctttttaaagcggaccaaatatgataacctgcacttggaagatttatttataggcaacaaagtgaatgtcttctctcgacaactggtattaattgactatggggatcaatatacagctcgccagctgggcagtaggaaagaaaaaacgctagccctaattaaaccagatgcaatatcaaaggctggagaaataattgaaataataaacaaagctggatttactataaccaaactcaaaatgatgatgctttcaaggaaagaagcattggattttcatgtagatcaccagtcaagaccctttttcaatgagctgatccagtttattacaactggtcctattattgccatggagattttaagagatgatgctatatgtgaatggaaaagactgctgggacctgcaaactctggagtggcacgcacagatgcttctgaaagcattagagccctctttggaacagatggcataagaaatgcagcgcatggccctgattcttttgcttctgcggccagagaaatggagttgttttttccttcaagtggaggttgtgggccggcaaacactgctaaatttactaattgtacctgttgcattgttaaaccccatgctgtcagtgaaggactgttgggaaagatcctgatggctatccgagatgcaggttttgaaatctcagctatgcagatgttcaatatggatcgggttaatgttgaggaattctatgaagtttataaaggagtagtgaccgaatatcatgacatggtgacagaaatgtattctggcccttgtgtagcaatggagattcaacagaataatgctacaaagacatttcgagaattttgtggacctgctgatcctgaaattgcccggcatttacgccctggaactctcagagcaatctttggtaaaactaagatccagaatgctgttcactgtactgatctgccagaggatggcctattagaggttcaatacttcttcaagatcttggataatacgcgtacgcggccgctcgagcagaaactcatctcagaagaggatctggcagcaaatgatatcctggattacaaggatgacgacgataaggtttaa

SEQ ID NO: 81 - protein, 407 aa, Artificial Sequence
  OriGene-NME7-1 full length
MNHSERFVFIAEWYDPNASLLRRYELLFYPGDGSVEMHDVKNHRTFLKRTKYDNLHLEDLFIGNKVNVFSRQLVLIDYGDQYTARQLGSRKEKTLALIKPDAISKAGEIIEIINKAGFTITKLKMMMLSRKEALDFHVDHQSRPFFNELIQFITTGPIIAMEILRDDAICEWKRLLGPANSGVARTDASESIRALFGTDGIRNAAHGPDSFASAAREMELFFPSSGGCGPANTAKFTNCTCCIVKPHAVSEGLLGKILMAIRDAGFEISAMQMFNMDRVNVEEFYEVYKGVVTEYHDMVTEMYSGPCVAMEIQQNNATKTFREFCGPADPEIARHLRPGTLRAIFGKTKIQNAVHCTDLPEDGLLEVQYFFKILDNTRTRRLEQKLISEEDLAANDILDYKDDDDKV

SEQ ID NO: 82 - protein, 376 aa, Artificial Sequence
  Abnova NME7-1 Full length
MNHSERFVFIAEWYDPNASLLRRYELLFYPGDGSVEMHDVKNHRTFLKRTKYDNLHLEDLFIGNKVNVFSRQLVLIDYGDQYTARQLGSRKEKTLALIKPDAISKAGEIIEIINKAGFTITKLKMMMLSRKEALDFHVDHQSRPFFNELIQFITTGPIIAMEILRDDAICEWKRLLGPANSGVARTDASESIRALFGTDGIRNAAHGPDSFASAAREMELFFPSSGGCGPANTAKFTNCTCCIVKPHAVSEGLLGKILMAIRDAGFEISAMQMFNMDRVNVEEFYEVYKGVVTEYHDMVTEMYSGPCVAMEIQQNNATKTFREFCGPADPEIARHLRPGTLRAIFGKTKIQNAVHCTDLPEDGLLEVQYFFKILDN

SEQ ID NO: 83 - protein, 98 aa, Artificial Sequence
  Abnova Partial NME7-B
DRVNVEEFYEVYKGVVTEYHDMVTEMYSGPCVAMEIQQNNATKTFREFCGPADPEIARHLRPGTLRAIFGKTKIQNAVHCTDLPEDGLLEVQYFFKIL

SEQ ID NO: 84 - DNA, 27 bp, Artificial Sequence
  Histidine Tag
ctcgagcaccaccaccaccaccactga

SEQ ID NO: 85 - protein, 36 aa, Artificial Sequence
  Strept II Tag
ACCGGTTGGAGCCATCCTCAGTTCGAAAAGTAATGA

SEQ ID NO: 86 - protein, 35 aa, Artificial Sequence
  N-10 peptide
QFNQYKTEAASRYNLTISDVSVSDVPFPFSAQSGA

SEQ ID NO: 87 - protein, 35 aa, Artificial Sequence
  C-10 peptide
GTINVHDVETQFNQYKTEAASRYNLTISDVSVSDV

SEQ ID NO: 88 - protein, 8 aa, Artificial Sequence
  C-10 peptide
LALIKPDA

SEQ ID NO: 89 - protein, 18 aa, Artificial Sequence
  C-10 peptide
MMMLSRKEALDFHVDHQS

SEQ ID NO: 90 - protein, 10 aa, Artificial Sequence
  C-10 peptide
ALDFHVDHQS

SEQ ID NO: 91 - protein, 14 aa, Artificial Sequence
  C-10 peptide
EILRDDAICEWKRL

SEQ ID NO: 92 - protein, 12 aa, Artificial Sequence
  C-10 peptide
FNELIQFITTGP

SEQ ID NO: 93 - protein, 8 aa, Artificial Sequence
  C-10 peptide
RDDAICEW

SEQ ID NO: 94 - protein, 25 aa, Artificial Sequence
  C-10 peptide
SGVARTDASESIRALFGTDGIRNAA

SEQ ID NO: 95 - protein, 9 aa, Artificial Sequence
  C-10 peptide
ELFFPSSGG

SEQ ID NO: 96 - protein, 26 aa, Artificial Sequence
  C-10 peptide
KFTNCTCCIVKPHAVSEGLLGKILMA

SEQ ID NO: 97 - protein, 36 aa, Artificial Sequence
  C-10 peptide
LMAIRDAGFEISAMQMFNMDRVNVEEFYEVYKGVVT

SEQ ID NO: 98 - protein, 15 aa, Artificial Sequence
  C-10 peptide
EFYEVYKGVVTEYHD

SEQ ID NO: 99 - protein, 43 aa, Artificial Sequence
  C-10 peptide
EIQQNNATKTFREFCGPADPEIARHLRPGTLRAIFGKTKIQNA

SEQ ID NO: 100 - protein, 8 aa, Artificial Sequence
  C-10 peptide
YSGPCVAM

SEQ ID NO: 101 - protein, 7 aa, Artificial Sequence
  C-10 peptide
FREFCGP

SEQ ID NO: 102 - protein, 23 aa, Artificial Sequence
  C-10 peptide
VHCTDLPEDGLLEVQYFFKILDN

SEQ ID NO: 103 - protein, 9 aa, Artificial Sequence
  C-10 peptide
IQNAVHCTD

SEQ ID NO: 104 - protein, 20 aa, Artificial Sequence
  C-10 peptide
TDLPEDGLLEVQYFFKILDN

SEQ ID NO: 105 - protein, 13 aa, Artificial Sequence
  C-10 peptide
PEDGLLEVQYFFK

SEQ ID NO: 106 - protein, 12 aa, Artificial Sequence
  C-10 peptide
EIINKAGFTITK

SEQ ID NO: 107 - protein, 16 aa, Artificial Sequence
  C-10 peptide
MLSRKEALDFHVDHQS

SEQ ID NO: 108 - protein, 9 aa, Artificial Sequence
  C-10 peptide
NELIQFITT

SEQ ID NO: 109 - protein, 14 aa, Artificial Sequence
  C-10 peptide
EILRDDAICEWKRL

SEQ ID NO: 110 - protein, 21 aa, Artificial Sequence
  C-10 peptide
SGVARTDASESIRALFGTDGI

SEQ ID NO: 111 - protein, 11 aa, Artificial Sequence
  C-10 peptide
SGVARTDASES

SEQ ID NO: 112 - protein, 8 aa, Artificial Sequence
  C-10 peptide
ALFGTDGI

SEQ ID NO: 113 - protein, 14 aa, Artificial Sequence
  C-10 peptide
NCTCCIVKPHAVSE

SEQ ID NO: 114 - protein, 11 aa, Artificial Sequence
  C-10 peptide
LGKILMAIRDA

SEQ ID NO: 115 - protein, 16 aa, Artificial Sequence
  C-10 peptide
EISAMQMFNMDRVNVE

SEQ ID NO: 116 - protein, 8 aa, Artificial Sequence
  C-10 peptide
EVYKGVVT

SEQ ID NO: 117 - protein, 8 aa, Artificial Sequence
  C-10 peptide
EYHDMVTE

SEQ ID NO: 118 - protein, 15 aa, Artificial Sequence
  C-10 peptide
EFCGPADPEIARHLR

SEQ ID NO: 119 - protein, 12 aa, Artificial Sequence
  C-10 peptide
AIFGKTKIQNAV

SEQ ID NO: 120 - protein, 18 aa, Artificial Sequence
  C-10 peptide
LPEDGLLEVQYFFKILDN

SEQ ID NO: 121 - protein, 17 aa, Artificial Sequence
  C-10 peptide
GPDSFASAAREMELFFP

SEQ ID NO: 122 - protein, 7 aa, Artificial Sequence
  Immunizing peptides derived from human NME7
ICEWKRL

SEQ ID NO: 123 - protein, 11 aa, Artificial Sequence
  Immunizing peptides derived from human NME7
LGKILMAIRDA

SEQ ID NO: 124 - protein, 10 aa, Artificial Sequence
  Immunizing peptides derived from human NME7
HAVSEGLLGK

SEQ ID NO: 125 - protein, 8 aa, Artificial Sequence
  Immunizing peptides derived from human NME7
VTEMYSGP

SEQ ID NO: 126 - protein, 9 aa, Artificial Sequence
  Immunizing peptides derived from human NME7
NATKTFREF

SEQ ID NO: 127 - protein, 9 aa, Artificial Sequence
  Immunizing peptides derived from human NME7
AIRDAGFEI

SEQ ID NO: 128 - protein, 13 aa, Artificial Sequence
  Immunizing peptides derived from human NME7
AICEWKRLLGPAN

SEQ ID NO: 129 - protein, 8 aa, Artificial Sequence
  Immunizing peptides derived from human NME7
DHQSRPFF

SEQ ID NO: 130 - protein, 13 aa, Artificial Sequence
  Immunizing peptides derived from human NME7
AICEWKRLLGPAN

SEQ ID NO: 131 - protein, 8 aa, Artificial Sequence
  Immunizing peptides derived from human NME7
VDHQSRPF

SEQ ID NO: 132 - protein, 6 aa, Artificial Sequence
  Immunizing peptides derived from human NME7
PDSFAS

SEQ ID NO: 133 - protein, 18 aa, Artificial Sequence
  Immunizing peptides derived from human NME7
KAGEIIEIINKAGFTITK

SEQ ID NO: 134 - protein, 29 aa, Artificial Sequence
  Immunizing peptides derived from human NME1
MANCERTFIAIKPDGVQRGLVGEIIKRFE

SEQ ID NO: 135 - protein, 8 aa, Artificial Sequence
  Immunizing peptides derived from human NME1
VDLKDRPF

SEQ ID NO: 136 - protein, 17 aa, Artificial Sequence
  Immunizing peptides derived from human NME1
HGSDSVESAEKEIGLWF

SEQ ID NO: 137 - protein, 25 aa, Artificial Sequence
  Immunizing peptides derived from human NME1
ERTFIAIKPDGVQRGLVGEIIKRFE

SEQ ID NO: 138 - protein, 30 aa, Artificial Sequence
  Immunizing peptides derived from human NME1
VDLKDRPFFAGLVKYMHSGPVVAMVWEGLN

SEQ ID NO: 139 - protein, 26 aa, Artificial Sequence
  Immunizing peptides derived from human NME1
NIIHGSDSVESAEKEIGLWFHPEELV

SEQ ID NO: 140 - protein, 14 aa, Artificial Sequence
  Immunizing peptides derived from human NME1
KPDGVQRGLVGEII

SEQ ID NO: 141 - protein, 152 aa, Artificial Sequence
  NME1, aka NME-H1
MANCERTFIAIKPDGVQRGLVGEIIKRFEQKGFRLVGLKFMQASEDLLKEHYVDLKDRPFFAGLVKYMHSGPVVAMVWEGLNVVKTGRVMLGETNPADSKPGTIRGDFCIQVGRNIIHGSDSVESAEKEIGLWFHPEELVDYTSCAQNWIYE

SEQ ID NO: 142 - protein, 141 aa, Artificial Sequence
  Halomonas Sp 593 bacterial NME
MATERTLSIIKPDAVAKNVIGEIESRFEKAGLKIVAAKMLQLSQEQAEGFYAEHKERPFFGDLVGFMTSGPVVVQVLEGENAIAANRDLMGATNPKEAEAGTIRADYAQSIDANAVHGSDSPESAAREIAYFFEESEICSR

SEQ ID NO: 143 - protein, 131 aa, Artificial Sequence
  NME7A
EKTLALIKPDAISKAGEIIEIINKAGFTITKLKMMMLSRKEALDFHVDHQSRPFFNELIQFITTGPIIAMEILRDDAICEWKRLLGPANSGVARTDASESIRALFGTDGIRNAAHGPDSFASAAREMELFF

SEQ ID NO: 144 - protein, 130 aa, Artificial Sequence
  Halomonas Sp 593 bacterial NME
ERTLSIIKPDAVAKNVIGEIESRFEKAGLKIVAAKMLQLSQEQAEGFYAEHKERPFFGDLVGFMTSGPVVVQVLEGENAIAANRDLMGATNPKEAEAGTIRADYAQSIDANAVHGSDSPESAAREIAYFF

SEQ ID NO: 145 - protein, 132 aa, Artificial Sequence
  NME7B
TCCIVKPHAVSEGLLGKILMAIRDAGFEISAMQMFNMDRVNVEEFYEVYKGVVTEYHDMVTEMYSGPCVAMEIQQNNATKTFREFCGPADPEIARHLRPGTLRAIFGKTKIQNAVHCTDLPEDGLLEVQYFF

SEQ ID NO: 146 - protein, 128 aa, Artificial Sequence
  Halomonas Sp 593 bacterial NME
TLSIIKPDAVAKNVIGEIESRFEKAGLKIVAAKMLQLSQEQAEGFYAEHKERPFFGDLVGFMTSGPVVVQVLEGENAIAANRDLMGATNPKEAEAGTIRADYAQSIDANAVHGSDSPESAAREIAYFF